European Patent Specification EP 3 172 325 B1, published June 28, 2023. Title: MOLECULAR CONSTRUCTS AND USES THEREOF. Applicant: The University of Notre Dame du Lac. The sequence listing filed with the application follows.

SEQUENCE LISTING (15 sequences)

SEQ ID NO: 1 - protein, 608 aa, Homo sapiens
MKSLRVLLVILWLQLSWVWSQQKEVEQNSGPLSVPEGAIASLNCTYSYRGSQSFFWYRQYSGKSPELIMFIYSNGDKEDGRFTAQLNKASQYVSLLIRDSQPSDSATYLCAVNFGGGKLIFGQGTELSVKPNIQNPDPAVYQLRDSKSSDKSVCLFTDFDSQTNVSQSKDSDVYITDKTVLDMRSMDFKSNSAVAWSNKSDFACANAFNNSIIPEDTFFPSPESSCDVKLVEKSFETDTNLNFQNLSVIGFRILLLKVAGFNLLMTLRLWSSTGGSGATNFSLLKQAGDVEENPGPGPRIRLLCCVAFSLLWAGPVIAGITQAPTSQILAAGRRMTLRCTQDMRHNAMYWYRQDLGLGLRLIHYSNTAGTTGKGEVPDGYSVSRANTDDFPLTLASAVPSQTSVYFCASSWSFGTEAFFGQGTRLTVVEDLNKVFPPEVAVFEPSEAEISHTQKATLVCLATGFFPDHVELSWWVNGKEVHSGVSTDPQPLKEQPALNDSRYCLSSRLRVSATFWQNPRNHFRCQVQFYGLSENDEWTQDRAKPVTQIVSAEAWGRADCGFTSVSYQQGVLSATILYEILLGKATLYAVLVSALVLMAMVKRKDFEFK

SEQ ID NO: 2 - protein, 608 aa, Homo sapiens
MKSLRVLLVILWLQLSWVWSQQKEVEQNSGPLSVPEGAIASLNCTYSYRGSQSFFWYRQYSGKSPELIMFIYSNGDKEDGRFTAQLNKASQYVSLLIRDSQPSDSATYLCAVNFGGGKLIFGQGTELSVKPNIQNPDPAVYQLRDSKSSDKSVCLFTDFDSQTNVSQSKDSDVYITDKTVLDMRSMDFKSNSAVAWSNKSDFACANAFNNSIIPEDTFFPSPESSCDVKLVEKSFETDTNLNFQNLSVIGFRILLLKVAGFNLLMTLRLWSSTGGSGATNFSLLKQAGDVEENPGPGPRIRLLCCVAFSLLWAGPVIAGITQAPTSQILAAGRRMTLRCTQDMRHNAMYWYRQDLGLGLRLIHYSNTAGTTGKGEVPDGYSVSRANTDDFPLTLASAVPSQTSVYFCASSLSFGTEAFFGQGTRLTVVEDLNKVFPPEVAVFEPSEAEISHTQKATLVCLATGFFPDHVELSWWVNGKEVHSGVSTDPQPLKEQPALNDSRYCLSSRLRVSATFWQNPRNHFRCQVQFYGLSENDEWTQDRAKPVTQIVSAEAWGRADCGFTSVSYQQGVLSATILYEILLGKATLYAVLVSALVLMAMVKRKDFEFK

SEQ ID NO: 3 - protein, 608 aa, Homo sapiens
MKSLRVLLVILWLQLSWVWSQQKEVEQNSGPLSVPEGAIASLNCTYSDRGSQSFFWYRQYSGKSPELIMFIYSNGDKEDGRFTAQLNKASQYVSLLIRDSQPSDSATYLCAVNFGGGKLIFGQGTELSVKPNIQNPDPAVYQLRDSKSSDKSVCLFTDFDSQTNVSQSKDSDVYITDKTVLDMRSMDFKSNSAVAWSNKSDFACANAFNNSIIPEDTFFPSPESSCDVKLVEKSFETDTNLNFQNLSVIGFRILLLKVAGFNLLMTLRLWSSTGGSGATNFSLLKQAGDVEENPGPGPRIRLLCCVAFSLLWAGPVIAGITQAPTSQILAAGRRMTLRCTQDMRHNAMYWYRQDLGLGLRLIHYSNTAGTTGKGEVPDGYSVSRANTDDFPLTLASAVPSQTSVYFCASSWSFGTEAFFGQGTRLTVVEDLNKVFPPEVAVFEPSEAEISHTQKATLVCLATGFFPDHVELSWWVNGKEVHSGVSTDPQPLKEQPALNDSRYCLSSRLRVSATFWQNPRNHFRCQVQFYGLSENDEWTQDRAKPVTQIVSAEAWGRADCGFTSVSYQQGVLSATILYEILLGKATLYAVLVSALVLMAMVKRKDFEFK

SEQ ID NO: 4 - protein, 608 aa, Homo sapiens
MKSLRVLLVILWLQLSWVWSQQKEVEQNSGPLSVPEGAIASLNCTYSDRGSQSFFWYRQYSGKSPELIMFIYSNGDKEDGRFTAQLNKASQYVSLLIRDSQPSDSATYLCAVNFGGGKLIFGQGTELSVKPNIQNPDPAVYQLRDSKSSDKSVCLFTDFDSQTNVSQSKDSDVYITDKTVLDMRSMDFKSNSAVAWSNKSDFACANAFNNSIIPEDTFFPSPESSCDVKLVEKSFETDTNLNFQNLSVIGFRILLLKVAGFNLLMTLRLWSSTGGSGATNFSLLKQAGDVEENPGPGPRIRLLCCVAFSLLWAGPVIAGITQAPTSQILAAGRRMTLRCTQDMRHNAMYWYRQDLGLGLRLIHYSNTAGTTGKGEVPDGYSVSRANTDDFPLTLASAVPSQTSVYFCASSLSFGTEAFFGQGTRLTVVEDLNKVFPPEVAVFEPSEAEISHTQKATLVCLATGFFPDHVELSWWVNGKEVHSGVSTDPQPLKEQPALNDSRYCLSSRLRVSATFWQNPRNHFRCQVQFYGLSENDEWTQDRAKPVTQIVSAEAWGRADCGFTSVSYQQGVLSATILYEILLGKATLYAVLVSALVLMAMVKRKDFEFK

SEQ ID NO: 5 - protein, 9 aa, Homo sapiens
AAGIGILTV

SEQ ID NO: 6 - protein, 608 aa, Homo sapiens
MKSLRVLLVILWLQLSWVWSQQKEVEQNSGPLSVPEGAIASLNCTYSYRGSQSFFWYRQYSGKSPELIMFIVSNGDKEDGRFTAQLNKASQYVSLLIRDSQPSDSATYLCAVNFGGGKLIFGQGTELSVKPNIQNPDPAVYQLRDSKSSDKSVCLFTDFDSQTNVSQSKDSDVYITDKTVLDMRSMDFKSNSAVAWSNKSDFACANAFNNSIIPEDTFFPSPESSCDVKLVEKSFETDTNLNFQNLSVIGFRILLLKVAGFNLLMTLRLWSSTGGSGATNFSLLKQAGDVEENPGPGPRIRLLCCVAFSLLWAGPVIAGITQAPTSQILAAGRRMTLRCTQDMRHNAMYWYRQDLGLGLRLIHYSNTAGTTGKGEVPDGYSVSRANTDDFPLTLASAVPSQTSVYFCASSLSFGTEAFFGQGTRLTVVEDLNKVFPPEVAVFEPSEAEISHTQKATLVCLATGFFPDHVELSWWVNGKEVHSGVSTDPQPLKEQPALNDSRYCLSSRLRVSATFWQNPRNHFRCQVQFYGLSENDEWTQDRAKPVTQIVSAEAWGRADCGFTSVSYQQGVLSATILYEILLGKATLYAVLVSALVLMAMVKRKDFEFK

SEQ ID NO: 7 - protein, 10 aa, Homo sapiens
ELAGIGILTV

SEQ ID NO: 8 - protein, 608 aa, Homo sapiens
MKSLRVLLVILWLQLSWVWSQQKEVEQNSGPLSVPEGAIASLNCTYSYRGSQSFFWYRQYSGKSPELIMFIASNGDKEDGRFTAQLNKASQYVSLLIRDSQPSDSATYLCAVNFGGGKLIFGQGTELSVKPNIQNPDPAVYQLRDSKSSDKSVCLFTDFDSQTNVSQSKDSDVYITDKTVLDMRSMDFKSNSAVAWSNKSDFACANAFNNSIIPEDTFFPSPESSCDVKLVEKSFETDTNLNFQNLSVIGFRILLLKVAGFNLLMTLRLWSSTGGSGATNFSLLKQAGDVEENPGPGPRIRLLCCVAFSLLWAGPVIAGITQAPTSQILAAGRRMTLRCTQDMRHNAMYWYRQDLGLGLRLIHYSNTAGTTGKGEVPDGYSVSRANTDDFPLTLASAVPSQTSVYFCASSWSFGTEAFFGQGTRLTVVEDLNKVFPPEVAVFEPSEAEISHTQKATLVCLATGFFPDHVELSWWVNGKEVHSGVSTDPQPLKEQPALNDSRYCLSSRLRVSATFWQNPRNHFRCQVQFYGLSENDEWTQDRAKPVTQIVSAEAWGRADCGFTSVSYQQGVLSATILYEILLGKATLYAVLVSALVLMAMVKRKDFEFK

SEQ ID NO: 9 - protein, 608 aa, Homo sapiens
MKSLRVLLVILWLQLSWVWSQQKEVEQNSGPLSVPEGAIASLNCTYSYRGSQSFFWYRQYSGKSPELIMFIVSNGDKEDGRFTAQLNKASQYVSLLIRDSQPSDSATYLCAVNFGGGKLIFGQGTELSVKPNIQNPDPAVYQLRDSKSSDKSVCLFTDFDSQTNVSQSKDSDVYITDKTVLDMRSMDFKSNSAVAWSNKSDFACANAFNNSIIPEDTFFPSPESSCDVKLVEKSFETDTNLNFQNLSVIGFRILLLKVAGFNLLMTLRLWSSTGGSGATNFSLLKQAGDVEENPGPGPRIRLLCCVAFSLLWAGPVIAGITQAPTSQILAAGRRMTLRCTQDMRHNAMYWYRQDLGLGLRLIHYSNTAGTTGKGEVPDGYSVSRANTDDFPLTLASAVPSQTSVYFCASSWSFGTEAFFGQGTRLTVVEDLNKVFPPEVAVFEPSEAEISHTQKATLVCLATGFFPDHVELSWWVNGKEVHSGVSTDPQPLKEQPALNDSRYCLSSRLRVSATFWQNPRNHFRCQVQFYGLSENDEWTQDRAKPVTQIVSAEAWGRADCGFTSVSYQQGVLSATILYEILLGKATLYAVLVSALVLMAMVKRKDFEFK

SEQ ID NO: 10 - protein, 608 aa, Homo sapiens
MKSLRVLLVILWLQLSWVWSQQKEVEQNSGPLSVPEGAIASLNCTYSYRGSQSFFWYRQYSGKSPELIMFIFSNGDKEDGRFTAQLNKASQYVSLLIRDSQPSDSATYLCAVNFGGGKLIFGQGTELSVKPNIQNPDPAVYQLRDSKSSDKSVCLFTDFDSQTNVSQSKDSDVYITDKTVLDMRSMDFKSNSAVAWSNKSDFACANAFNNSIIPEDTFFPSPESSCDVKLVEKSFETDTNLNFQNLSVIGFRILLLKVAGFNLLMTLRLWSSTGGSGATNFSLLKQAGDVEENPGPGPRIRLLCCVAFSLLWAGPVIAGITQAPTSQILAAGRRMTLRCTQDMRHNAMYWYRQDLGLGLRLIHYSNTAGTTGKGEVPDGYSVSRANTDDFPLTLASAVPSQTSVYFCASSWSFGTEAFFGQGTRLTVVEDLNKVFPPEVAVFEPSEAEISHTQKATLVCLATGFFPDHVELSWWVNGKEVHSGVSTDPQPLKEQPALNDSRYCLSSRLRVSATFWQNPRNHFRCQVQFYGLSENDEWTQDRAKPVTQIVSAEAWGRADCGFTSVSYQQGVLSATILYEILLGKATLYAVLVSALVLMAMVKRKDFEFK

SEQ ID NO: 11 - protein, 608 aa, Homo sapiens
MKSLRVLLVILWLQLSWVWSQQKEVEQNSGPLSVPEGAIASLNCTYSYRGSQSFFWYRQYSGKSPELIMFIWSNGDKEDGRFTAQLNKASQYVSLLIRDSQPSDSATYLCAVNFGGGKLIFGQGTELSVKPNIQNPDPAVYQLRDSKSSDKSVCLFTDFDSQTNVSQSKDSDVYITDKTVLDMRSMDFKSNSAVAWSNKSDFACANAFNNSIIPEDTFFPSPESSCDVKLVEKSFETDTNLNFQNLSVIGFRILLLKVAGFNLLMTLRLWSSTGGSGATNFSLLKQAGDVEENPGPGPRIRLLCCVAFSLLWAGPVIAGITQAPTSQILAAGRRMTLRCTQDMRHNAMYWYRQDLGLGLRLIHYSNTAGTTGKGEVPDGYSVSRANTDDFPLTLASAVPSQTSVYFCASSWSFGTEAFFGQGTRLTVVEDLNKVFPPEVAVFEPSEAEISHTQKATLVCLATGFFPDHVELSWWVNGKEVHSGVSTDPQPLKEQPALNDSRYCLSSRLRVSATFWQNPRNHFRCQVQFYGLSENDEWTQDRAKPVTQIVSAEAWGRADCGFTSVSYQQGVLSATILYEILLGKATLYAVLVSALVLMAMVKRKDFEFK

SEQ ID NO: 12 - protein, 10 aa, Homo sapiens
EAAGIGILTV

SEQ ID NO: 13 - protein, 605 aa, Homo sapiens
MKSLRVLLVILWLQLSWVWSQQKEVEQNSGPLSVPEGAIASLNCTYSDRGSQSFFWYRQYSGKSPELIMFIYSNGDKEDGRFTAQLNKASQYVSLLIRDSQPSDSATYLCAVNFGGGKLIFGQGTELSVKPNIQNPDPAVYQLRDSKSSDKSVCLFTDFDSQTNVSQSKDSDVYITDKTVLDMRSMDFKSNSAVAWSNKSDFACANAFNNSIIPEDTFFPSPESSCDVKLVEKSFETDTNLNFQNLSVIGFRILLLKVAGFNLLMTLRLWSSTGGSGATNFSLLKQAGDVEENPGPGPRIRLLCCVAFSLLWAGPVIAGITQAPTSQILAAGRRMTLRCTQDMRHNAMYWYRQDLGLGLRLIHYSNTAGTTGKGEVPDGYSVSRANTDDFPLTLASAVPSQTSVYFCASSLSFGTEAFFGQGTRLTVVEDLNKVFPPEVAVFEPSEAEISHTQKATLVCLATGFFPDHVELSWWVNGKEVHSGVSTDPQPLKEQPALNDSRYCLSSRLRVSATFWQNPRNHFRCQVQFYGLSENDEWTQDRAKPVTQIVSAEAWGRADCGFTSVSYQQGVLSATILYEILLGKATLYAVLVSALVLMAMVKRKDF

SEQ ID NO: 14 - DNA, 1859 bp, Homo sapiens
aaagcggccgctacgtagtcgactgcacctagaatatgaaatccttgagagttttactagtgatcctgtggcttcagttgagctgggtttggagccaacagaaggaggtggagcagaactctggacccctcagtgttccagagggagccattgcctctctcaactgcacttacagtgaccgaggttcccagtccttcttctggtacagacaatattctgggaaaagccctgagttgataatgttcatatactccaatggtgacaaagaagatggaaggtttacagcacagctcaataaagccagccagtatgtttctctgctcatcagagactcccagcccagtgattcagccacctacctctgtgccgtgaacttcggaggaggaaagcttatcttcggacagggaacggagctatctgtgaaacccaatatccagaaccctgaccctgccgtgtaccagctgagagactctaaatccagtgacaagtctgtctgcctattcaccgattttgattctcaaacaaatgtgtcacaaagtaaggattctgatgtgtatatcacagacaaaactgtgctagacatgaggtctatggacttcaagagcaacagtgctgtggcctggagcaacaaatctgactttgcatgtgcaaacgccttcaacaacagcattattccagaagacaccttcttccccagcccagaaagttcctgtgatgtcaagctggtcgagaaaagctttgaaacagatacgaacctaaactttcaaaacctgtcagtgattgggttccgaatcctcctcctgaaagtggccgggtttaatctgctcatgacgctgcggctgtggtccagcaccggtgggtccggagccacgaacttctctctgttaaagcaagcaggagacgtggaggagaaccccggtcctgggcccagaatcaggctcctgtgctgtgtggccttttctctcctgtgggcaggtccagtgattgctgggatcacccaggcaccaacatctcagatcctggcagcaggacggcgcatgacactgagatgtacccaggatatgagacataatgccatgtactggtatagacaagatctaggactggggctaaggctcatccattattcaaatactgcaggtaccactggcaaaggagaagtccctgatggttatagtgtctccagagcaaacacagatgatttccccctcacgttggcgtctgctgtaccctctcagacatctgtgtacttctgtgccagcagtttgtccttcggaactgaagctttctttggacaaggcaccagactcacagttgtagaggacctgaacaaggtgttcccacccgaggtcgctgtgtttgagccatcagaagcagagatctcccacacccaaaaggccacactggtgtgcctggccacaggcttcttccccgaccacgtggagctgagctggtgggtgaatgggaaggaggtgcacagtggggtcagcacggacccgcagcccctcaaggagcagcccgccctcaatgactccagatactgcctgagcagccgcctgagggtctcggccaccttctggcagaacccccgcaaccacttccgctgtcaagtccagttctacgggctctcggagaatgacgagtggacccaggatagggccaaacccgtcacccagatcgtcagcgccgaggcctggggtagagcagactgtggctttacctcggtgtcctaccagcaaggggtcctgtctgccaccatcctctatgagatcctgctagggaaggccaccctgtatgctgtgctggtcagcgcccttgtgttgatggccatggtcaagagaaaggatttcgaattcaaa

SEQ ID NO: 15 - protein, 586 aa, Synthetic Sequence
  featureMiscellaneous (50)..(50): Xaa is any amino acid except tyrosine
KEVEQNSGPLSVPEGAIASLNCTYSYRGSQSFFWYRQYSGKSPELIMFIXSNGDKEDGRFTAQLNKASQYVSLLIRDSQPSDSATYLCAVNFGGGKLIFGQGTELSVKPNIQNPDPAVYQLRDSKSSDKSVCLFTDFDSQTNVSQSKDSDVYITDKTVLDMRSMDFKSNSAVAWSNKSDFACANAFNNSIIPEDTFFPSPESSCDVKLVEKSFETDTNLNFQNLSVIGFRILLLKVAGFNLLMTLRLWSSTGGSGATNFSLLKQAGDVEENPGPGPRIRLLCCVAFSLLWAGPVIAGITQAPTSQILAAGRRMTLRCTQDMRHNAMYWYRQDLGLGLRLIHYSNTAGTTGKGEVPDGYSVSRANTDDFPLTLASAVPSQTSVYFCASSWSFGTEAFFGQGTRLTVVEDLNKVFPPEVAVFEPSEAEISHTQKATLVCLATGFFPDHVELSWWVNGKEVHSGVSTDPQPLKEQPALNDSRYCLSSRLRVSATFWQNPRNHFRCQVQFYGLSENDEWTQDRAKPVTQIVSAEAWGRADCGFTSVSYQQGVLSATILYEILLGKATLYAVLVSALVLMAMVKRKDFEFK